European Patent Application EP 4 166 945 A1, published April 19, 2023. Title: Novel Biomarkers of Membranous Glomerulonephritis. Applicant: Universitätsklinikum Hamburg-Eppendorf. The sequence listing filed with the application follows.

SEQUENCE LISTING (10 sequences)

SEQ ID NO: 1 - protein, 539 aa, Homo sapiens
MYLSRFLSIHALWVTVSSVMQPYPLVWGHYDLCKTQIYTEEGKVWDYMACQPESTDMTKYLKVKLDPPDITCGDPPETFCAMGNPYMCNNECDASTPELAHPPELMFDFEGRHPSTFWQSATWKEYPKPLQVNITLSWSKTIELTDNIVITFESGRPDQMILEKSLDYGRTWQPYQYYATDCLDAFHMDPKSVKDLSQHTVLEIICTEEYSTGYTTNSKIIHFEIKDRFAFFAGPRLRNMASLYGQLDTTKKLRDFFTVTDLRIRLLRPAVGEIFVDELHLARYFYAISDIKVRGRCKCNLHATVCVYDNSKLTCECEHNTTGPDCGKCKKNYQGRPWSPGSYLPIPKGTANTCIPSISSIGNCECFGHSNRCSYIDLLNTVICVSCKHNTRGQHCELCRLGYFRNASAQLDDENVCIECYCNPLGSIHDRCNGSGFCECKTGTTGPKCDECLPGNSWHYGCQPNVCDNELLHCQNGGTCHNNVRCLCPAAYTGILCEKLRCEEAGSCGSDSGQGAPPHGSPALLLLTTLLGTASPLVF

SEQ ID NO: 2 - protein, 510 aa, Homo sapiens
MYLSRFLSIHALWVTVSSVMQPYPLVWGHYDLCKTQIYTEEGKVWDYMACQPESTDMTKYLKVKLDPPDITCGDPPETFCAMGNPYMCNNECDASTPELAHPPELMFDFEGRHPSTFWQSATWKEYPKPLQVNITLSWSKTIELTDNIVITFESGRPDQMILEKSLDYGRTWQPYQYYATDCLDAFHMDPKSVKDLSQHTVLEIICTEEYSTGYTTNSKIIHFEIKDRFAFFAGPRLRNMASLYGQLDTTKKLRDFFTVTDLRIRLLRPAVGEIFVDELHLARYFYAISDIKVRGRCKCNLHATVCVYDNSKLTCECEHNTTGPDCGKCKKNYQGRPWSPGSYLPIPKGTANTCIPSISSIGNCECFGHSNRCSYIDLLNTVICVSCKHNTRGQHCELCRLGYFRNASAQLDDENVCIECYCNPLGSIHDRCNGSGFCECKTGTTGPKCDECLPGNSWHYGCQPNVCDNELLHCQNGGTCHNNVRCLCPAAYTGILCEKLRCEEAGSCGS

SEQ ID NO: 3 - protein, 482 aa, Homo sapiens
HYDLCKTQIYTEEGKVWDYMACQPESTDMTKYLKVKLDPPDITCGDPPETFCAMGNPYMCNNECDASTPELAHPPELMFDFEGRHPSTFWQSATWKEYPKPLQVNITLSWSKTIELTDNIVITFESGRPDQMILEKSLDYGRTWQPYQYYATDCLDAFHMDPKSVKDLSQHTVLEIICTEEYSTGYTTNSKIIHFEIKDRFAFFAGPRLRNMASLYGQLDTTKKLRDFFTVTDLRIRLLRPAVGEIFVDELHLARYFYAISDIKVRGRCKCNLHATVCVYDNSKLTCECEHNTTGPDCGKCKKNYQGRPWSPGSYLPIPKGTANTCIPSISSIGNCECFGHSNRCSYIDLLNTVICVSCKHNTRGQHCELCRLGYFRNASAQLDDENVCIECYCNPLGSIHDRCNGSGFCECKTGTTGPKCDECLPGNSWHYGCQPNVCDNELLHCQNGGTCHNNVRCLCPAAYTGILCEKLRCEEAGSCGS

SEQ ID NO: 4 - DNA, 1620 bp, Homo sapiens
atgtatttgtcaagattcctgtcgattcatgccctttgggttacggtgtcctcagtgatgcagccctaccctttggtttggggacattatgatttgtgtaagactcagatttacacggaagaagggaaagtttgggattacatggcctgccagccggaatccacggacatgacaaaatatctgaaagtgaaactcgatcctccggatattacctgtggagaccctcctgagacgttctgtgcaatgggcaatccctacatgtgcaataatgagtgtgatgcgagtacccctgagctggcacacccccctgagctgatgtttgattttgaaggaagacatccctccacattttggcagtctgccacttggaaggagtatcccaagcctctccaggttaacatcactctgtcttggagcaaaaccattgagctaacagacaacatagttattacctttgaatctgggcgtccagaccaaatgatcctggagaagtctctcgattatggacgaacatggcagccctatcagtattatgccacagactgcttagatgcttttcacatggatcctaaatccgtgaaggatttatcacagcatacggtcttagaaatcatttgcacagaagagtactcaacagggtatacaacaaatagcaaaataatccactttgaaatcaaagacaggttcgcgttttttgctggacctcgcctacgcaatatggcttccctctacggacagctggatacaaccaagaaactcagagatttctttacagtcacagacctgaggataaggctgttaagaccagccgttggggaaatatttgtagatgagctacacttggcacgctacttttacgcgatctcagacataaaggtgcgaggaaggtgcaagtgtaatctccatgccactgtatgtgtgtatgacaacagcaaattgacatgcgaatgtgagcacaacactacaggtccagactgtgggaaatgcaagaagaattatcagggccgaccttggagtccaggctcctatctccccatccccaaaggcactgcaaatacctgtatccccagtatttccagtattggtaattgtgaatgcttcggccactccaatcgatgcagttatatcgatctgctaaatacagtcatttgcgtgagctgtaaacacaacactagagggcagcactgtgagttatgcaggctgggctacttcagaaatgcttctgcacaactggacgatgagaatgtgtgcatagagtgttattgtaaccctttgggctcaatccatgatcgttgtaatggctcaggattttgtgagtgtaagactggaacaacagggcctaagtgtgatgagtgtctgccgggaaattcctggcactacggctgtcaaccgaatgtctgcgacaacgagctcctgcactgccagaacggagggacgtgccacaacaacgtgcgctgcctgtgcccggccgcatacacgggcatcctctgcgagaagctgcggtgcgaggaggctggcagctgcggctccgactctggccagggcgcgcccccgcacggctccccagcgctgctgctgctgaccacgctgctgggaaccgccagccccctggtgttctag

SEQ ID NO: 5 - protein, 438 aa, Homo sapiens
MYLSRFLSIHALWVTVSSVMQPYPLVWGHYDLCKTQIYTEEGKVWDYMACQPESTDMTKYLKVKLDPPDITCGDPPETFCAMGNPYMCNNECDASTPELAHPPELMFDFEGRHPSTFWQSATWKEYPKPLQVNITLSWSKTIELTDNIVITFESGRPDQMILEKSLDYGRTWQPYQYYATDCLDAFHMDPKSVKDLSQHTVLEIICTEEYSTGYTTNSKIIHFEIKDRFAFFAGPRLRNMASLYGQLDTTKKLRDFFTVTDLRIRLLRPAVGEIFVDELHLARYFYAISDIKVRGRCKCNLHATVCVYDNSKLTCECEHNTTGPDCGKCKKNYQGRPWSPGSYLPIPKGTANTCIPSISSIGTNVCDNELLHCQNGGTCHNNVRCLCPAAYTGILCEKLRCEEAGSCGSDSGQGAPPHGSPALLLLTTLLGTASPLVF

SEQ ID NO: 6 - protein, 364 aa, Homo sapiens
MYLSRFLSIHALWVTVSSVMQPYPLVWGHYDLCKTQIYTEEGKVWDYMACQPESTDMTKYLKVKLDPPDITCGDPPETFCAMGNPYMCNNECDASTPELAHPPELMFDFEGRHPSTFWQSATWKEYPKPLQVNITLSWSKTIELTDNIVITFESGRPDQMILEKSLDYGRTWQPYQYYATDCLDAFHMDPKSVKDLSQHTVLEIICTEEYSTGYTTNSKIIHFEIKDRFAFFAGPRLRNMASLYGQLDTTKKLRDFFTVTDLRIRLLRPAVGEIFVDELHLARYFYAISDIKVRGRCKCNLHATVCVYDNSKLTCECEHNTTGPDCGKCKKNYQGRPWSPGSYLPIPKGTANTCIPSISSIGSK

SEQ ID NO: 7 - protein, 480 aa, Homo sapiens
MYLSRFLSIHALWVTVSSVMQPYPLVWGHYDLCKTQIYTEEGKVWDYMACQPESTDMTKYLKVKLDPPDITCGDPPETFCAMGNPYMCNNECDASTPELAHPPELMFDFEGRHPSTFWQSATWKEYPKPLQVNITLSWSKTIELTDNIVITFESGRPDQMILEKSLDYGRTWQPYQYYATDCLDAFHMDPKSVKDLSQHTVLEIICTEEYSTGYTTNSKIIHFEIKDRFAFFAGPRLRNMASLYGQLDTTKKLRDFFTVTDLRIRLLRPAVGEIFVDELHLARYFYAISDIKVRGRCKCNLHATVCVYDNSKLTCECEHNTTGPDCGKCKKNYQGRPWSPGSYLPIPKGTANTCIPSISSIGNPPKFNRIWPNISSLEVSNPKQVAPKLALSTVSSVQVANHKRANVCDNELLHCQNGGTCHNNVRCLCPAAYTGILCEKLRCEEAGSCGSDSGQGAPPHGSPALLLLTTLLGTASPLVF

SEQ ID NO: 8 - protein, 460 aa, Homo sapiens
MYLSRFLSIHALWVTVSSVMQPYPLVWGHYDLCKTQIYTEEGKVWDYMACQPESTDMTKYLKVKLDPPDITCGDPPETFCAMGNPYMCNNECDASTPELAHPPELMFDFEGRHPSTFWQSATWKEYPKPLQVNITLSWSKTIELTDNIVITFESGRPDQMILEKSLDYGRTWQPYQYYATDCLDAFHMDPKSVKDLSQHTVLEIICTEEYSTGYTTNSKIIHFEIKDRFAFFAGPRLRNMASLYGQLDTTKKLRDFFTVTDLRIRLLRPAVGEIFVDELHLARYFYAISDIKVRGRCKCNLHATVCVYDNSKLTCECEHNTTGPDCGKCKKNYQGRPWSPGSYLPIPKGTANTCIPSISSIGNPPKFNRIWPNISSLEVSNPKQANVCDNELLHCQNGGTCHNNVRCLCPAAYTGILCEKLRCEEAGSCGSDSGQGAPPHGSPALLLLTTLLGTASPLVF

SEQ ID NO: 9 - protein, 1462 aa, Homo sapiens
MLLSPSLLLLLLLGAPRGCAEGVAAALTPERLLEWQDKGIFVIQSESLKKCIQAGKSVLTLENCKQANKHMLWKWVSNHGLFNIGGSGCLGLNFSAPEQPLSLYECDSTLVSLRWRCNRKMITGPLQYSVQVAHDNTVVASRKYIHKWISYGSGGGDICEYLHKDLHTIKGNTHGMPCMFPFQYNHQWHHECTREGREDDLLWCATTSRYERDEKWGFCPDPTSAEVGCDTIWEKDLNSHICYQFNLLSSLSWSEAHSSCQMQGGTLLSITDETEENFIREHMSSKTVEVWMGLNQLDEHAGWQWSDGTPLNYLNWSPEVNFEPFVEDHCGTFSSFMPSAWRSRDCESTLPYICKKYLNHIDHEIVEKDAWKYYATHCEPGWNPYNRNCYKLQKEEKTWHEALRSCQADNSALIDITSLAEVEFLVTLLGDENASETWIGLSSNKIPVSFEWSNDSSVIFTNWHTLEPHIFPNRSQLCVSAEQSEGHWKVKNCEERLFYICKKAGHVLSDAESGCQEGWERHGGFCYKIDTVLRSFDQASSGYYCPPALVTITNRFEQAFITSLISSVVKMKDSYFWIALQDQNDTGEYTWKPVGQKPEPVQYTHWNTHQPRYSGGCVAMRGRHPLGRWEVKHCRHFKAMSLCKQPVENQEKAEYEERWPFHPCYLDWESEPGLASCFKVFHSEKVLMKRTWREAEAFCEEFGAHLASFAHIEEENFVNELLHSKFNWTEERQFWIGFNKRNPLNAGSWEWSDRTPVVSSFLDNTYFGEDARNCAVYKANKTLLPLHCGSKREWICKIPRDVKPKIPFWYQYDVPWLFYQDAEYLFHTFASEWLNFEFVCSWLHSDLLTIHSAHEQEFIHSKIKALSKYGASWWIGLQEERANDEFRWRDGTPVIYQNWDTGRERTVNNQSQRCGFISSITGLWGSEECSVSMPSICKRKKVWLIEKKKDTPKQHGTCPKWLYFNYKCLLLNIPKDPSSWKNWTHAQHFCAEEGGTLVAIESEVEQAFITMNLFGQTTSVWIGLQNDDYETWLNGKPVVYSNWSPFDIINIPSHNTTEVQKHIPLCALLSSNPNFHFTGKWYFEDCGKEGYGFVCEKMQDTSGHGVNTSDMYPMPNTLEYGNRTYKIINANMTWYAAIKTCLMHKAQLVSITDQYHQSFLTVVLNRLGYAHWIGLFTTDNGLNFDWSDGTKSSFTFWKDEESSLLGDCVFADSNGRWHSTACESFLQGAICHVPPETRQSEHPELCSETSIPWIKFKSNCYSFSTVLDSMSFEAAHEFCKKEGSNLLTIKDEAENAFLLEELFAFGSSVQMVWLNAQFDGNNETIKWFDGTPTDQSNWGIRKPDTDYFKPHHCVALRIPEGLWQLSPCQEKKGFICKMEADIHTAEALPEKGPSHSIIPLAVVLTLIVIVAICTLSFCIYKHNGGFFRRLAGFRNPYYPATNFSTVYLEENILISDLEKSDQ

SEQ ID NO: 10 - protein, 1656 aa, Homo sapiens
MGLQARRWASGSRGAAGPRRGVLQLLPLPLPLPLLLLLLLRPGAGRAAAQGEAEAPTLYLWKTGPWGRCMGDECGPGGIQTRAVWCAHVEGWTTLHTNCKQAERPNNQQNCFKVCDWHKELYDWRLGPWNQCQPVISKSLEKPLECIKGEEGIQVREIACIQKDKDIPAEDIICEYFEPKPLLEQACLIPCQQDCIVSEFSAWSECSKTCGSGLQHRTRHVVAPPQFGGSGCPNLTEFQVCQSSPCEAEELRYSLHVGPWSTCSMPHSRQVRQARRRGKNKEREKDRSKGVKDPEARELIKKKRNRNRQNRQENKYWDIQIGYQTREVMCINKTGKAADLSFCQQEKLPMTFQSCVITKECQVSEWSEWSPCSKTCHDMVSPAGTRVRTRTIRQFPIGSEKECPEFEEKEPCLSQGDGVVPCATYGWRTTEWTECRVDPLLSQQDKRRGNQTALCGGGIQTREVYCVQANENLLSQLSTHKNKEASKPMDLKLCTGPIPNTTQLCHIPCPTECEVSPWSAWGPCTYENCNDQQGKKGFKLRKRRITNEPTGGSGVTGNCPHLLEAIPCEEPACYDWKAVRLGNCEPDNGKECGPGTQVQEVVCINSDGEEVDRQLCRDAIFPIPVACDAPCPKDCVLSTWSTWSSCSHTCSGKTTEGKQIRARSILAYAGEEGGIRCPNSSALQEVRSCNEHPCTVYHWQTGPWGQCIEDTSVSSFNTTTTWNGEASCSVGMQTRKVICVRVNVGQVGPKKCPESLRPETVRPCLLPCKKDCIVTPYSDWTSCPSSCKEGDSSIRKQSRHRVIIQLPANGGRDCTDPLYEEKACEAPQACQSYRWKTHKWRRCQLVPWSVQQDSPGAQEGCGPGRQARAITCRKQDGGQAGIHECLQYAGPVPALTQACQIPCQDDCQLTSWSKFSSCNGDCGAVRTRKRTLVGKSKKKEKCKNSHLYPLIETQYCPCDKYNAQPVGNWSDCILPEGKVEVLLGMKVQGDIKECGQGYRYQAMACYDQNGRLVETSRCNSGYIEEACIIPCPSDCKLSEWSNWSRCSKSCGSGVKVRSKWLREKPYNGGRPCPKLDHVNQAQVYEVVPCHSDCNQYLWVTEPWSICKVTFVNMRENCGEGVQTRKVRCMQNTADGPSEHVEDYLCDPEEMPLGSRVCKLPCPEDCVISEWGPWTQCVLPCNQSSFRQRSADPIRQPADEGRSCPNAVEKEPCNLNKNCYHYDYNVTDWSTCQLSEKAVCGNGIKTRMLDCVRSDGKSVDLKYCEALGLEKNWQMNTSCMVECPVNCQLSDWSPWSECSQTCGLTGKMIRRRTVTQPFQGDGRPCPSLMDQSKPCPVKPCYRWQYGQWSPCQVQEAQCGEGTRTRNISCVVSDGSADDFSKVVDEEFCADIELIIDGNKNMVLEESCSQPCPGDCYLKDWSSWSLCQLTCVNGEDLGFGGIQVRSRPVIIQELENQHLCPEQMLETKSCYDGQCYEYKWMASAWKGSSRTVWCQRSDGINVTGGCLVMSQPDADRSCNPPCSQPHSYCSETKTCHCEEGYTEVMSSNSTLEQCTLIPVVVLPTMEDKRGDVKTSRAVHPTQPSSNPAGRGRTWFLQPFGPDGRLKTWVYGVAAGAFVLLIFIVSMIYLACKKPKKPQRRQNNRLKPLTLAYDGDADM